European Patent Specification EP 3 211 004 B1, published December 6, 2023. Title: Use of Macrophage inflammatory protein-1 (MIP-1) inhibitor for improving tissue ischemia and diabetes vasculopathy by promoting angiogenesis. Applicant: Farmar Licensing Co., Ltd. Chen, Jaw-Wen. Application 15 852 326.6. The sequence listing filed with the application follows.

SEQUENCE LISTING (2 sequences)

SEQ ID NO: 1 - protein, 9 aa, Mus musculus
SFVMDYYET

SEQ ID NO: 2 - protein, 13 aa, Mus musculus
AVVFLTKRGRQIC